European Patent Application EP 4 389 767 A1, published June 26, 2024. Title: 靶向SIRPα的单克隆抗体及其用途. Applicant: 杭州九源基因工程有限公司. The sequence listing filed with the application follows.

SEQUENCE LISTING (44 sequences)

SEQ ID NO: 1 - protein, 571 aa, synthetic construct
EEELQVIQPDKSVLVAAGETATLRCTATSLIPVGPIQWFRGAGPGRELIYNQKEGHFPRVTTVSDLTKRNNMDFSIRIGNITPADAGTYYCVKFRKGSPDDVEFKSGAGTELSVRAKPSAPVVSGPAARATPQHTVSFTCESHGFSPRDITLKWFKNGNELSDFQTNVDPVGESVSYSIHSTAKVVLTREDVHSQVICEVAHVTLQGDPLRGTANLSETIRVPPTLEVTQQPVRAENQVNVTCQVRKFYPQRLQLTWLENGNVSRTETASTVTENKDGTYNWMSWLLVNVSAHRDDVKLTCQVEHDGQPAVSKSHDLKVSAHPKEQGSNTAAENTGSNERPKSCLKTHTCPPCPAPELLGGPSVFLFPPKPKDTLMISRTPEVTCVVVDVSHEDPEVKFNWYVDGVEVHNAKTKPREEQYNSTYRVVSVLTVLHQDWLNGKEYKCKVSNKALPAPIEKTISKAKGQPREPQVYTLPPSRDELTKNQVSLTCLVKGFYPSDIAVEWESNGQPENNYKTTPPVLDSDGSFFLYSKLTVDKSRWQQGNVFSCSVMHEALHNHYTQKSLSLSPGK

SEQ ID NO: 2 - protein, 474 aa, synthetic construct
EEELQVIQPDKSVLVAAGETATLRCTATSLIPVGPIQWFRGAGPGRELIYNQKEGHFPRVTTVSDLTKRNNMDFSIRIGNITPADAGTYYCVKFRKGSPDDVEFKSGAGTELSVRAKPSAPVVSGPAARATPQHTVSFTCESHGFSPRDITLKWFKNGNELSDFQTNVDPVGESVSYSIHSTAKVVLTREDVHSQVICEVAHVTLQGDPLRGTANLSETIRVPPTLEVTQQPVRAENQVNVTCQVRKFYPQRLQLTWLENGNVSRTETASTVTENKDGTYNWMSWLLVNVSAHRDDVKLTCQVEHDGQPAVSKSHDLKVSAHPKEQGSNTAAENTGSNERNIYIVVGVVCTLLVALLMAALYLVRIRQKKAQGSTSSTRLHEPEKNAREITQDTNDITYADLNLPKGKKPAPQAAEPNNHTEYASIQTSPQPASEDTLTYADLDMVHLNRTPKQPAPKPEPSFSEYASVQVPRK

SEQ ID NO: 3 - protein, 114 aa, synthetic construct
EVQLEESGPGLVAPSQSLSITCTVSGFSLTGYGVNWVRQPPGKGLEWLGIIWGDGSTDYNSALKSRLSISKDNSKSQVFLKMNSLQSDDTARYYCARAGKMDYWGQGTSVTVSS

SEQ ID NO: 4 - protein, 111 aa, synthetic construct
DIVLTQSPASLAVSLGQGATISCRASESVDSYGNSFMHWYQQKPGQPPKPLIYLASNLESGVPARFSGSGSRTDFTLTIDPVEADDAATYYCQQNNEYPWTFGGGTKLEIK

SEQ ID NO: 5 - protein, 10 aa, synthetic construct
GFSLTGYGVN

SEQ ID NO: 6 - protein, 16 aa, synthetic construct
IIWGDGSTDYNSALKS

SEQ ID NO: 7 - protein, 6 aa, synthetic construct
AGKMDY

SEQ ID NO: 8 - protein, 14 aa, synthetic construct
RASESVDSYGNSFM

SEQ ID NO: 9 - protein, 7 aa, synthetic construct
LASNLES

SEQ ID NO: 10 - protein, 9 aa, synthetic construct
QQNNEYPWT

SEQ ID NO: 11 - protein, 114 aa, synthetic construct
QVQLQESGPGLVKPSQTLSLTCTVSGFSLTGYGVNWIRQPPGKGLEWIGIIWGDASTDYNAALKSRVTISKDTSKNQVFLKLSSVTAADTAVYYCARAGKMDYWGQGTTVTVSS

SEQ ID NO: 12 - protein, 111 aa, synthetic construct
DIVLTQSPASLAVSPGQRATITCRASESVDSYGNSFMHWYQQKPGQPPKPLIYLASNLESGVPARFSGSGSGTDFTLTINPVEANDAANYYCQQNNEYPWTFGGGTKVEIK

SEQ ID NO: 13 - protein, 232 aa, synthetic construct
EPKSCDKTHTCPPCPAPEAAGGPSVFLFPPKPKDTLMISRTPEVTCVVVDVSHEDPEVKFNWYVDGVEVHNAKTKPREEQYNSTYRVVSVLTVLHQDWLNGKEYKCKVSNKALPAPIEKTISKAKGQPREPQVYTLPPSRDELTKNQVSLTCLVKGFYPSDIAVEWESNGQPENNYKTTPPVLDSDGSFFLYSKLTVDKSRWQQGNVFSCSVMHEALHNHYTQKSLSLSPGK

SEQ ID NO: 14 - protein, 16 aa, synthetic construct
IIWGDASTDYNAALKS

SEQ ID NO: 15 - protein, 114 aa, synthetic construct
QVQLQESGPGLVKPSQTLSLTCTVSGFSLTGYGVNWIRQPPGKGLEWIGIIWGDGSTDYNSALKSRVTISVDTSKNQFSLKLSSVTAADTAVYYCARAGKMDYWGQGTTVTVSS

SEQ ID NO: 16 - protein, 114 aa, synthetic construct
QVQLQESGPGLVKPSQTLSLTCTVSGFSLTGYGVNWIRQPPGKGLEWIGIIWGDGSTDYNSALKSRVTISVDTSKNQVFLKLSSVTAADTAVYYCARAGKMDYWGQGTTVTVSS

SEQ ID NO: 17 - protein, 114 aa, synthetic construct
QVQLQESGPGLVKPSQTLSLTCTVSGFSLTGYGVNWIRQPPGKGLEWIGIIWGDGSTDYNSALKSRVTISKDTSKNQVFLKLSSVTAADTAVYYCARAGKMDYWGQGTTVTVSS

SEQ ID NO: 18 - protein, 114 aa, synthetic construct
QVQLQESGPGLVKPSQTLSLTCTVSGFSLTGYGVNWIRQPPGKGLEWIGIIWGDGSTDYNSALKSRVTISKDTSKNQVFLKLSSVTADDTARYYCARAGKMDYWGQGTTVTVSS

SEQ ID NO: 19 - protein, 111 aa, synthetic construct
DIVLTQSPASLAVSPGQRATITCRASESVDSYGNSFMHWYQQKPGQPPKLLIYLASNLESGVPARFSGSGSGTDFTLTINPVEANDTANYYCQQNNEYPWTFGGGTKVEIK

SEQ ID NO: 20 - protein, 111 aa, synthetic construct; identical to SEQ ID NO: 12

SEQ ID NO: 21 - protein, 111 aa, synthetic construct
DIVLTQSPASLAVSPGQRATITCRASESVDSYGNSFMHWYQQKPGQPPKLLIYLASNLESGVPARFSGSGSRTDFTLTINPVEANDAANYYCQQNNEYPWTFGGGTKVEIK

SEQ ID NO: 22 - protein, 111 aa, synthetic construct
DIVLTQSPASLAVSPGQRATITCRASESVDSYGNSFMHWYQQKPGQPPKPLIYLASNLESGVPARFSGSGSRTDFTLTINPVEANDAANYYCQQNNEYPWTFGGGTKVEIK

SEQ ID NO: 23 - protein, 16 aa, synthetic construct
IIWGDASTDYNSALKS

SEQ ID NO: 24 - protein, 16 aa, synthetic construct
IIWGDGSTDYNAALKS

SEQ ID NO: 25 - protein, 14 aa, synthetic construct
RASESVDSYGSSFM

SEQ ID NO: 26 - protein, 218 aa, synthetic construct
DIVLTQSPASLAVSPGQRATITCRASESVDSYGSSFMHWYQQKPGQPPKPLIYLASNLESGVPARFSGSGSGTDFTLTINPVEANDAANYYCQQNNEYPWTFGGGTKVEIKRTVAAPSVFIFPPSDEQLKSGTASVVCLLNNFYPREAKVQWKVDNALQSGNSQESVTEQDSKDSTYSLSSTLTLSKADYEKHKVYACEVTHQGLSSPVTKSFNRGEC

SEQ ID NO: 27 - protein, 218 aa, synthetic construct
DIVLTQSPASLAVSPGQRATITCRASESVDSYGNSFMHWYQQKPGQPPKPLIYLASNLESGVPARFSGSGSGTDFTLTINPVEANDAANYYCQQNNEYPWTFGGGTKVEIKRTVAAPSVFIFPPSDEQLKSGTASVVCLLNNFYPREAKVQWKVDNALQSGNSQESVTEQDSKDSTYSLSSTLTLSKADYEKHKVYACEVTHQGLSSPVTKSFNRGEC

SEQ ID NO: 28 - protein, 444 aa, synthetic construct
QVQLQESGPGLVKPSQTLSLTCTVSGFSLTGYGVNWIRQPPGKGLEWIGIIWGDGSTDYNSALKSRVTISKDTSKNQVFLKLSSVTAADTAVYYCARAGKMDYWGQGTTVTVSSASTKGPSVFPLAPSSKSTSGGTAALGCLVKDYFPEPVTVSWNSGALTSGVHTFPAVLQSSGLYSLSSVVTVPSSSLGTQTYICNVNHKPSNTKVDKKVEPKSCDKTHTCPPCPAPEAAGGPSVFLFPPKPKDTLMISRTPEVTCVVVDVSHEDPEVKFNWYVDGVEVHNAKTKPREEQYNSTYRVVSVLTVLHQDWLNGKEYKCKVSNKALPAPIEKTISKAKGQPREPQVYTLPPSRDELTKNQVSLTCLVKGFYPSDIAVEWESNGQPENNYKTTPPVLDSDGSFFLYSKLTVDKSRWQQGNVFSCSVMHEALHNHYTQKSLSLSPGK

SEQ ID NO: 29 - protein, 444 aa, synthetic construct
QVQLQESGPGLVKPSQTLSLTCTVSGFSLTGYGVNWIRQPPGKGLEWIGIIWGDASTDYNSALKSRVTISKDTSKNQVFLKLSSVTAADTAVYYCARAGKMDYWGQGTTVTVSSASTKGPSVFPLAPSSKSTSGGTAALGCLVKDYFPEPVTVSWNSGALTSGVHTFPAVLQSSGLYSLSSVVTVPSSSLGTQTYICNVNHKPSNTKVDKKVEPKSCDKTHTCPPCPAPEAAGGPSVFLFPPKPKDTLMISRTPEVTCVVVDVSHEDPEVKFNWYVDGVEVHNAKTKPREEQYNSTYRVVSVLTVLHQDWLNGKEYKCKVSNKALPAPIEKTISKAKGQPREPQVYTLPPSRDELTKNQVSLTCLVKGFYPSDIAVEWESNGQPENNYKTTPPVLDSDGSFFLYSKLTVDKSRWQQGNVFSCSVMHEALHNHYTQKSLSLSPGK

SEQ ID NO: 30 - protein, 444 aa, synthetic construct
QVQLQESGPGLVKPSQTLSLTCTVSGFSLTGYGVNWIRQPPGKGLEWIGIIWGDGSTDYNAALKSRVTISKDTSKNQVFLKLSSVTAADTAVYYCARAGKMDYWGQGTTVTVSSASTKGPSVFPLAPSSKSTSGGTAALGCLVKDYFPEPVTVSWNSGALTSGVHTFPAVLQSSGLYSLSSVVTVPSSSLGTQTYICNVNHKPSNTKVDKKVEPKSCDKTHTCPPCPAPEAAGGPSVFLFPPKPKDTLMISRTPEVTCVVVDVSHEDPEVKFNWYVDGVEVHNAKTKPREEQYNSTYRVVSVLTVLHQDWLNGKEYKCKVSNKALPAPIEKTISKAKGQPREPQVYTLPPSRDELTKNQVSLTCLVKGFYPSDIAVEWESNGQPENNYKTTPPVLDSDGSFFLYSKLTVDKSRWQQGNVFSCSVMHEALHNHYTQKSLSLSPGK

SEQ ID NO: 31 - protein, 444 aa, synthetic construct
QVQLQESGPGLVKPSQTLSLTCTVSGFSLTGYGVNWIRQPPGKGLEWIGIIWGDASTDYNAALKSRVTISKDTSKNQVFLKLSSVTAADTAVYYCARAGKMDYWGQGTTVTVSSASTKGPSVFPLAPSSKSTSGGTAALGCLVKDYFPEPVTVSWNSGALTSGVHTFPAVLQSSGLYSLSSVVTVPSSSLGTQTYICNVNHKPSNTKVDKKVEPKSCDKTHTCPPCPAPEAAGGPSVFLFPPKPKDTLMISRTPEVTCVVVDVSHEDPEVKFNWYVDGVEVHNAKTKPREEQYNSTYRVVSVLTVLHQDWLNGKEYKCKVSNKALPAPIEKTISKAKGQPREPQVYTLPPSRDELTKNQVSLTCLVKGFYPSDIAVEWESNGQPENNYKTTPPVLDSDGSFFLYSKLTVDKSRWQQGNVFSCSVMHEALHNHYTQKSLSLSPGK

SEQ ID NO: 32 - protein, 330 aa, synthetic construct [sequence omitted]

SEQ ID NO: 33 - protein, 326 aa, synthetic construct
ASTKGPSVFPLAPCSRSTSESTAALGCLVKDYFPEPVTVSWNSGALTSGVHTFPAVLQSSGLYSLSSVVTVPSSNFGTQTYTCNVDHKPSNTKVDKTVERKCCVECPPCPAPPVAGPSVFLFPPKPKDTLMISRTPEVTCVVVDVSHEDPEVQFNWYVDGVEVHNAKTKPREEQFNSTFRVVSVLTVVHQDWLNGKEYKCKVSNKGLPAPIEKTISKTKGQPREPQVYTLPPSREEMTKNQVSLTCLVKGFYPSDIAVEWESNGQPENNYKTTPPMLDSDGSFFLYSKLTVDKSRWQQGNVFSCSVMHEALHNHYTQKSLSLSPGK

SEQ ID NO: 34 - protein, 327 aa, synthetic construct
ASTKGPSVFPLAPCSRSTSESTAALGCLVKDYFPEPVTVSWNSGALTSGVHTFPAVLQSSGLYSLSSVVTVPSSSLGTKTYTCNVDHKPSNTKVDKRVESKYGPPCPPCPAPEFLGGPSVFLFPPKPKDTLMISRTPEVTCVVVDVSQEDPEVQFNWYVDGVEVHNAKTKPREEQFNSTYRVVSVLTVLHQDWLNGKEYKCKVSNKGLPSSIEKTISKAKGQPREPQVYTLPPSQEEMTKNQVSLTCLVKGFYPSDIAVEWESNGQPENNYKTTPPVLDSDGSFFLYSRLTVDKSRWQEGNVFSCSVMHEALHNHYTQKSLSLSLGK

SEQ ID NO: 35 - protein, 444 aa, synthetic construct
QVQLQESGPGLVKPSQTLSLTCTVSGFSLTGYGVNWIRQPPGKGLEWIGIIWGDASTDYNAALKSRVTISKDTSKNQVFLKLSSVTAADTAVYYCARAGKMDYWGQGTTVTVSSASTKGPSVFPLAPSSKSTSGGTAALGCLVKDYFPEPVTVSWNSGALTSGVHTFPAVLQSSGLYSLSSVVTVPSSSLGTQTYICNVNHKPSNTKVDKKVEPKSCDKTHTCPPCPAPELLGGPSVFLFPPKPKDTLMISRTPEVTCVVVDVSHEDPEVKFNWYVDGVEVHNAKTKPREEQYNSTYRVVSVLTVLHQDWLNGKEYKCKVSNKALPAPIEKTISKAKGQPREPQVYTLPPSRDELTKNQVSLTCLVKGFYPSDIAVEWESNGQPENNYKTTPPVLDSDGSFFLYSKLTVDKSRWQQGNVFSCSVMHEALHNHYTQKSLSLSPGK

SEQ ID NO: 36 - protein, 440 aa, synthetic construct
QVQLQESGPGLVKPSQTLSLTCTVSGFSLTGYGVNWIRQPPGKGLEWIGIIWGDASTDYNAALKSRVTISKDTSKNQVFLKLSSVTAADTAVYYCARAGKMDYWGQGTTVTVSSASTKGPSVFPLAPCSRSTSESTAALGCLVKDYFPEPVTVSWNSGALTSGVHTFPAVLQSSGLYSLSSVVTVPSSNFGTQTYTCNVDHKPSNTKVDKTVERKCCVECPPCPAPPVAGPSVFLFPPKPKDTLMISRTPEVTCVVVDVSHEDPEVQFNWYVDGVEVHNAKTKPREEQFNSTFRVVSVLTVVHQDWLNGKEYKCKVSNKGLPAPIEKTISKTKGQPREPQVYTLPPSREEMTKNQVSLTCLVKGFYPSDIAVEWESNGQPENNYKTTPPMLDSDGSFFLYSKLTVDKSRWQQGNVFSCSVMHEALHNHYTQKSLSLSPGK

SEQ ID NO: 37 - protein, 441 aa, synthetic construct
QVQLQESGPGLVKPSQTLSLTCTVSGFSLTGYGVNWIRQPPGKGLEWIGIIWGDASTDYNAALKSRVTISKDTSKNQVFLKLSSVTAADTAVYYCARAGKMDYWGQGTTVTVSSASTKGPSVFPLAPCSRSTSESTAALGCLVKDYFPEPVTVSWNSGALTSGVHTFPAVLQSSGLYSLSSVVTVPSSSLGTKTYTCNVDHKPSNTKVDKRVESKYGPPCPPCPAPEFLGGPSVFLFPPKPKDTLMISRTPEVTCVVVDVSQEDPEVQFNWYVDGVEVHNAKTKPREEQFNSTYRVVSVLTVLHQDWLNGKEYKCKVSNKGLPSSIEKTISKAKGQPREPQVYTLPPSQEEMTKNQVSLTCLVKGFYPSDIAVEWESNGQPENNYKTTPPVLDSDGSFFLYSRLTVDKSRWQEGNVFSCSVMHEALHNHYTQKSLSLSLGK

SEQ ID NO: 38 - protein, 503 aa, synthetic construct
MEPAGPAPGRLGPLLCLLLAASCAWSGVAGEEELQVIQPDKSVSVAAGESAILHCTVTSLIPVGPIQWFRGAGPARELIYNQKEGHFPRVTTVSESTKRENMDFSISISNITPADAGTYYCVKFRKGSPDTEFKSGAGTELSVRAKPSAPVVSGPAARATPQHTVSFTCESHGFSPRDITLKWFKNGNELSDFQTNVDPVGESVSYSIHSTAKVVLTREDVHSQVICEVAHVTLQGDPLRGTANLSETIRVPPTLEVTQQPVRAENQVNVTCQVRKFYPQRLQLTWLENGNVSRTETASTVTENKDGTYNWMSWLLVNVSAHRDDVKLTCQVEHDGQPAVSKSHDLKVSAHPKEQGSNTAAENTGSNERNIYIVVGVVCTLLVALLMAALYLVRIRQKKAQGSTSSTRLHEPEKNAREITQDTNDITYADLNLPKGKKPAPQAAEPNNHTEYASIQTSPQPASEDTLTYADLDMVHLNRTPKQPAPKPEPSFSEYASVQVPRK

SEQ ID NO: 39 - protein, 503 aa, synthetic construct
MEPAGPAPGRLGPLLCLLLAASCAWSGVAGEEELQVIQPDKSVLVAAGETATLRCTATSLIPVGPIQWFRGAGPARELIYNQKEGHFPRVTTVSESTKRENMDFSISISNITPADAGTYYCVKFRKGSPDTEFKSGAGTELSVRAKPSAPVVSGPAARATPQHTVSFTCESHGFSPRDITLKWFKNGNELSDFQTNVDPVGESVSYSIHSTAKVVLTREDVHSQVICEVAHVTLQGDPLRGTANLSETIRVPPTLEVTQQPVRAENQVNVTCQVRKFYPQRLQLTWLENGNVSRTETASTVTENKDGTYNWMSWLLVNVSAHRDDVKLTCQVEHDGQPAVSKSHDLKVSAHPKEQGSNTAAENTGSNERNIYIVVGVVCTLLVALLMAALYLVRIRQKKAQGSTSSTRLHEPEKNAREITQDTNDITYADLNLPKGKKPAPQAAEPNNHTEYASIQTSPQPASEDTLTYADLDMVHLNRTPKQPAPKPEPSFSEYASVQVPRK

SEQ ID NO: 40 - protein, 121 aa, synthetic construct
QLLFNKTKSVEFTFCNDTVVIPCFVTNMEAQNTTEVYVKWKFKGRDIYTFDGALNKSTVPTDFSSAKIEVSQLLKGDASLKMDKSDAVSHTGNYTCEVTELTREGETIIELKYRVVSWFSP

SEQ ID NO: 41 - protein, 16 aa, synthetic construct
IIWGXXSTDYXXALKS

SEQ ID NO: 42 - protein, 14 aa, synthetic construct
RASESVDSYGXXFM

SEQ ID NO: 43 - protein, 16 aa, synthetic construct
IIWGDXSTDYNXALKS

SEQ ID NO: 44 - protein, 14 aa, synthetic construct
RASESVDSYGXSFM